European Patent Application EP 4 647 445 A1, published November 12, 2025. Title: ANTIGEN-BINDING PROTEIN TARGETING ROR1. Applicant: SPH BIOTHERAPEUTICS (SHANGHAI) LIMITED. The sequence listing filed with the application follows.

SEQUENCE LISTING (31 sequences)

SEQ ID NO: 1 - protein, 8 aa, synthetic construct
  REGION 1..8: note = 5-26/hu5-26 CDR1
GFTLDLYA

SEQ ID NO: 2 - protein, 7 aa, synthetic construct
  REGION 1..7: note = 5-26/hu5-26 CDR2
ISSGGST

SEQ ID NO: 3 - protein, 19 aa, synthetic construct
  REGION 1..19: note = 5-26 CDR3
VRSVPSCGSYPPFYRNMNY

SEQ ID NO: 4 - protein, 25 aa, synthetic construct
  REGION 1..25: note = 5-26/4-92 FR1
QVQLQESGGGLVQPGGSLRLSCAAS

SEQ ID NO: 5 - protein, 17 aa, synthetic construct
  REGION 1..17: note = 5-26 FR2
IGWFRQAPGKERERVSC

SEQ ID NO: 6 - protein, 38 aa, synthetic construct
  REGION 1..38: note = 5-26 FR3
NYAESVKGRFTISRDNGKNTVYLQMNSLKPEDTAVYYC

SEQ ID NO: 7 - protein, 11 aa, synthetic construct
  REGION 1..11: note = 5-26 FR4
WGKGTQVTVSS

SEQ ID NO: 8 - protein, 125 aa, synthetic construct
  REGION 1..125: note = 5-26 VHH
QVQLQESGGGLVQPGGSLRLSCAASGFTLDLYAIGWFRQAPGKERERVSCISSGGSTNYAESVKGRFTISRDNGKNTVYLQMNSLKPEDTAVYYCVRSVPSCGSYYFPPRNMNYWGKGTQVTVSS

SEQ ID NO: 9 - protein, 139 aa, synthetic construct
  REGION 1..139: note = VHH1
QVQLVESGGGLVQPGGSLRLSCAASGFTFSDTWMNWVRQAPGKGLYWISAINPDGGNTAYADSVKGRFTISRDNAKNMVYLQMDNLRPEDTAMYYCAKGWVRLPDPDLVRGQGTQVTVSSAAAYPYDVPDYGSHHHHHH

SEQ ID NO: 10 - protein, 144 aa, synthetic construct
  REGION 1..144: note = VHH2
QVQLVESGGGLVQAGGSLRLSCAASGSIFSINAMAWYRHRPGMQRERVAAISSGGTTSYADSVKGRFTISRDNARDTLYLQMNSLKPEDTAMYYCAACPGDYTSTICNSDGMDYWGKGTLVTVSSAAAYPYDVPDYGSHHHHHH

SEQ ID NO: 11 - protein, 125 aa, synthetic construct
  REGION 1..125: note = 5-9VHH
QVQLQESGGGLVQPGGSLRLSCAASGFTLDDYAIGWFRQAPGKERERISCISSGGNTNYADSVKGRFTLSRDNAKNTVYLQMYSLKPEDTAVYYCTASIPSCASYYFPPRNMDYWGKGTQVTVSS

SEQ ID NO: 12 - protein, 117 aa, synthetic construct
  REGION 1..117: note = 5-95VHH
QVQLQESGGGLVQPGGSLRLSCAASGFTFSTYSMTWVRQAPGKGLEWVSDINSGGSVAYYTDSVKGRFTASRDNAKNTLYLQMNSLKPEDTAVYYCYEGGYHGGSPRGHGTQVTVSS

SEQ ID NO: 13 - protein, 19 aa, synthetic construct
  REGION 1..19: note = hu5-26 CDR3-2
VRSVPSCGSYYFPPRNMNY

SEQ ID NO: 14 - protein, 25 aa, synthetic construct
  REGION 1..25: note = hu5-26 FR1
QVQLVESGGGLVQPGGSLRLSCAAS

SEQ ID NO: 15 - protein, 17 aa, synthetic construct
  REGION 1..17: note = hu5-26 FR2
IGWFRQAPGKERGLVSC

SEQ ID NO: 16 - protein, 38 aa, synthetic construct
  REGION 1..38: note = hu5-26 FR3
NYAESVKGRFTISRDNSKNTVYLQMNSLRSEDTAVYYC

SEQ ID NO: 17 - protein, 11 aa, synthetic construct
  REGION 1..11: note = hu5-26 FR4
WGQGTLVTVSS

SEQ ID NO: 18 - protein, 125 aa, synthetic construct
  REGION 1..125: note = hu5-26 VHH
QVQLVESGGGLVQPGGSLRLSCAASGFTLDLYAIGWFRQAPGKERGLVSCISSGGSTNYAESVKGRFTISRDNSKNTVYLQMNSLRSEDTAVYYCVRSVPSCGSYYFPPRNMNYWGQGTLVTVSS

SEQ ID NO: 19 - protein, 8 aa, synthetic construct
  REGION 1..8: note = 4-92 CDR1
GFAFSSRA

SEQ ID NO: 20 - protein, 8 aa, synthetic construct
  REGION 1..8: note = 4-92 CDR2
INYDGAWT

SEQ ID NO: 21 - protein, 8 aa, synthetic construct
  REGION 1..8: note = 4-92 CDR3
TDPWSIDG

SEQ ID NO: 22 - protein, 17 aa, synthetic construct
  REGION 1..17: note = 4-92 FR2
MSWVRQAPGKGLEWVSD

SEQ ID NO: 23 - protein, 38 aa, synthetic construct
  REGION 1..38: note = 4-92 FR3
YYADSVKGRFTISRDNAKNTLYLQMNSLKPEDTAVYFC

SEQ ID NO: 24 - protein, 11 aa, synthetic construct
  REGION 1..11: note = 4-92 FR4
WGQGTQVTVSS

SEQ ID NO: 25 - protein, 115 aa, synthetic construct
  REGION 1..115: note = 4-92 VHH
QVQLQESGGGLVQPGGSLRLSCAASGFAFSSRAMSWVRQAPGKGLEWVSDINYDGAWTYYADSVKGRFTISRDNAKNTLYLQMNSLKPEDTAVYFCTDPWSIDGWGQGTQVTVSS

SEQ ID NO: 26 - protein, 21 aa, synthetic construct
  REGION 1..21: note = CD8 SP
MALPVTALLLPLALLLHAARP

SEQ ID NO: 27 - protein, 39 aa, synthetic construct
  REGION 1..39: note = CD28 hinge region
IEVMYPPPYLDNEKSNGTIIHVKGKHLCPSPLFPGPSKP

SEQ ID NO: 28 - protein, 27 aa, synthetic construct
  REGION 1..27: note = CD28 transmembrane region
FWVLVVVGGVLACYSLLVTVAFIIFWV

SEQ ID NO: 29 - protein, 42 aa, synthetic construct
  REGION 1..42: note = 4-1BB
KRGRKKLLYIFKQPFMRPVQTTQEEDGCSCRFPEEEEGGCEL

SEQ ID NO: 30 - protein, 112 aa, synthetic construct
  REGION 1..112: note = CD3z
RVKFSRSADAPAYKQGQNQLYNELNLGRREEYDVLDKRRGRDPEMGGKPRRKNPQEGLYNELQKDKMAEAYSEIGMKGERRRGKGHDGLYQGLSTATKDTYDALHMQALPPR

SEQ ID NO: 31 - protein, 385 aa, synthetic construct
  REGION 1..385: note = CAR
MALPVTALLLPLALLLHAARPMGWSCIILFLVATATGVHSQVQLVESGGGLVQPGGSLRLSCAASGFTLDLYAIGWFRQAPGKERGLVSCISSGGSTNYAESVKGRFTISRDNSKNTVYLQMNSLRSEDTAVYYCVRSVPSCGSYYFPPRNMNYWGQGTLVTVSSIEVMYPPPYLDNEKSNGTIIHVKGKHLCPSPLFPGPSKPFWVLVVVGGVLACYSLLVTVAFIIFWVKRGRKKLLYIFKQPFMRPVQTTQEEDGCSCRFPEEEEGGCELRVKFSRSADAPAYKQGQNQLYNELNLGRREEYDVLDKRRGRDPEMGGKPRRKNPQEGLYNELQKDKMAEAYSEIGMKGERRRGKGHDGLYQGLSTATKDTYDALHMQALPPR